European Patent Specification EP 3 666 900 B1, published June 24, 2026. Title: CELL-BASED PRODUCTION OF NONULOSONATES. Applicant: National Research Council of Canada University of Ottawa. The sequence listing filed with the application follows.

SEQUENCE LISTING (48 sequences)

SEQ ID NO: 1 - protein, 333 aa, H. pylori
MPNHQNMLDNQTILITGGTGSFGKCFVRKVLDTTNAKKIIVYSRDELKQSEMAMEFNDPRMRFFIGDVRDLERLNYALEGVDICIHAAALKHVPIAEYNPLECIKTNIMGASNVINACLKNAISQVIALSTDKAANPINLYGATKLCSDKLFVSANNFKGSSQTQFSVVRYGNVVGSRGSVVPFFKKLVQNKASEIPITDIRMTRFWITLDEGVSFVLKSLKRMHGGEIFVPKIPSMKMTDLAKALAPNTPTKIIGIRPGEKLHEVMIPKDESHLALEFEDFFIIQPTISFQTPKDYTLTKLHEKGQKVAPDFEYSSHNNNQWLEPDDLLKLL

SEQ ID NO: 2 - protein, 375 aa, H. pylori
MKEFAYSEPCLDKEDKKAVLEVLNSKQLTQGKRSLLFEEALCEFLGVKHALVFNSATSALLTLYRNFSEFSADRNEIITTPISFVATANMLLESGYTPVFAGIKNDGNIDELALEKLINERTKAIVSVDYAGKSVEVESVQKLCKKHSLSFLSDSSHALGSEYQNKKVGGFALASVFSFHAIKPITTAEGGAVVTNDSELHEKMKLFRSHGMLKKDFFEGEVKSIGHNFRLNEIQSALGLSQLKKAPFLMQKREEAALTYDRIFKDNPYFTPLHPLLKDKSSNHLYPILMHQKFFTCKKLILESLHKRGILAQVHYKPIYQYQLYQQLFNTAPLKSAEDFYHAEISLPCHANLNLESVQNIAHSVLKTFESFKIE

SEQ ID NO: 3 - protein, 180 aa, H. pylori
MKKNYSYKNIQAIDFTNLNDGEKLLVLEFRNHPNTALWMYSTFISLKTHLQFIEDLKNSPNHRYFLFKEEGVYLGVGSITKINFFHKHGYLGIYKNPFLKNGGETILKALEFIAFEEFQLHSLHLEVMENNFKAIAFYEKNHYELEGRLKGFISKDKEFIDVLLYYKDKKGYNDQSLLKL

SEQ ID NO: 4 - protein, 340 aa, H. pylori
MLQPPKIVAELSANHNQDLNLAKESLHAIKESGADFVKLQTYTPSCMTLNSKEDPFIIQGTLWDKENLYELYQKASTPLEWHAELFELARKLDLGIFSSPFSSQALELLESLNCPMYKIASFEIVDLDLIEKAARTQKPIILSSGIATHTELQDAISLCRRVNNFDITLLKCVSAYPSKIEDANLLSMVKLGEIFGVKFGLSDHTIGSLCPILATTLGASMIEKHFILNKSLQTPDSAFSMDFNGFKSMVEAIKQSVLALGEEEPRINPKTLEKRRFFARSLFVIKDIQKGEALTENNIKALRPNLGLHPKFYKEILGQKASKFLKANTPLSADDIERSL

SEQ ID NO: 5 - protein, 274 aa, C. jejuni
MKVLFRSDSSSQIGFGHIKRDLVLAKQYSDVSFACLPLEGSLIDEIPYPVYELSSESIYELINLIKEEKFELLIIDHYGISVDDEKLIKLETGVKILSFDDEIKPHHCDILLNVNAYAKASDYEGLVPFKCEVRCGFSYALIREEFYQEAKENREKKYDFFICMGGTDIKNLSLQIASELPKTKIISIATSSSNPNLKKLQKFAKLHNNIRLFIDHENIAKLMNESNKLIISASSLVNEALLLKANFKAICYVKNQESTATWLAKKGYEVEYKY

SEQ ID NO: 6 - protein, 590 aa, C. jejuni
MIFYKSKRLAFFLTSDIVLILLSVYLAFSLRFSGDIPSIFYHGMMVSAIILLVLKLSFLFVFRIYKVAWRFFSLNEARKIFIALLLAEFCFFLIFYFFSDFFNPFPRSAIVIDFVLSYMFIGTLRISKRMLVDFKPSRMKEEETPCIVVGATSKALHLLKGAKEGSLGLFPVGVVDARKELIGTYCDKFIVEEKEKIKSYVEQGVKTAIIALRLEQEELKKLFEELVAYGICDVKIFSFTRNEARDISIEDLLARKPKDLDDSAVAAFLKDKVVLVSGAGGTIGSELCKQCIKFGAKHLIMVDHSEYNLYKINDDLNLYKEKITPILLSILDKQSLDEVLKTYKPELILHAAAYKHVPLCEQNPHSAVINNILGTKILCDSAKENKVAKFVMISTDKAVRPTNIMGCTKRVCELYTLSMSDENFEVACVRFGNVLGSSGSVIPKFKAQIANNEPLTLTHPDIVRYFMLVAEAVQLVLQAGAIAKGGELFVLDMGKPVKIIDLAKKMLLLSNRNDLEIKITGLRKGEKLYEELLIDENDAKTQYESIFVAKNEKVDLDWLNKEIENLQICEDISEALLKIVPEFKHNKEGV

SEQ ID NO: 7 - protein, 386 aa, C. jejuni
MRFFLSPPHMGGNELKYIEEVFKSNYIAPLGEFVNRFEQSVKAYSKSENALALNSATAALHLALRVAGVKQDDIVLASSFTFIASVAPICYLKAKPVFIDCDETYNIDVDLLKLAIKECEKKPKALILTHLYGNAAKMDEIVEICKENEIVLIEDAAEALGSFYKNKALGTFGEFGAYSYNGNKIITTSGGGMLIGKNKEKIEKARFYSTQARENCLHYEHLDYGYNYRLSNVLGAIGVAQMEVLEQRVLKKREIYEWYKEFLGECFSFLDELENSRSNRWLSTALIDFDKNELNSCQKDINISQKNITLHPKISKLIEDLKNEQIETRPLWKAMHAQEVFKGAKAYLNGNSELFFQKGICLPSGTAMSKDDVYEISKLILKSIKA

SEQ ID NO: 8 - protein, 195 aa, C. jejuni
MARTEKIYIYGASGHGLVCEDVAKNMGYKECIFLDDFKGMKFESTLPKYDFFIAIGNNEIRKKIYQKISENGFKIVNLIHKSALISPSAIVEENAGILIMPYVVINAKAKIEKGVILNTSSVIEHECVIGEFSHVSVGAKCAGNVKIGKNCFLGINSCVLPNLSLADDSILGGGATLVKNQDEKGVFVGVPAKRM

SEQ ID NO: 9 - protein, 334 aa, C. jejuni
MKKTLIIAEAGVNHNGDLNLAKKLIEIAADSGADFVKFQSFKAKNCISTKAKKAPYQLKTTANDESQLQMVQKLELDLKAHKELILHAKKCNIAFLSTPFDLESVDLLNELGLKIFKIPSGEITNLPYLKKIAKLNKKIILSTGMANLGEIEEALNVLCKNGAKRQNITLLHCTTEYPAPFNEVNLKAMQSLKDAFKLDVGYSDHTRGIHISLAAVALGACVIEKHFTLDKNMSGPDHKASLEPQELKMLCTQIRQIQKAMGDGIKKASKSEQKNINIVRKSLVAKKDIKKGEIFSEGNLTTKRPANGISAMRYEEFLGKIATKNYKEDELIRE

SEQ ID NO: 10 - protein, 356 aa, L. pneumophila
MGSNRKINGIKPRGSSMTCFIIAEAGVNHNGDLQLAKELVYAAKESGADAVKFQTFKADTLVNKTVEKAEYQKNNAPESSTQYEMLKALELSEEDHYLLSELANSLGIEFMSTGFDEQSIDFLISLGVKRLKIPSGEITNVPYLQHCASKKLPLIISTGMCDLQEVRVAIDTVKPYYGNSLSDYLVLLHCTSNYPASYQDVNLKAMQTLADEFQLPVGYSDHTLGILVPTLAVGMGACVIEKHFTMDKSLPGPDHLASMDPEEMKNLVQSIRDAETVLGSGEKKPSDNELPIRALVRRSITLRRDLVKGAQISKEDLILLRPGTGIAPSEISNIVGSRLSMNLSAGTTLLWEHIEA

SEQ ID NO: 11 - protein, 377 aa, L. pneumophila
MIRKIIYVTGTRADYGLMREVLKRLHQSEDIDLSICVTGMHLDALYGNTVNEIKADQFSICGIIPVDLANAQHSSMAKAIGHELLGFTEVFESETPDVVLLLGDRGEMLAAAIAAIHLNIPVVHLHGGERSGTVDEMVRHAISKLSHYHFVATEASKQRLIRMGEKEETIFQVGAPGLDEIMQYKTSTRDVFNQRYGFDPDKKICLLIYHPVVQEVDSIKIQFQSVIQAALATNLQIICLEPNSDTGGHLIREVIQEYIDHPDVRIIKHLHRPEFIDCLANSDVMLGNSSSGIIEAASFNLNVVNVGSRQNLRERSDNVIDVDVTYDAILTGLREALNKPKIKYSNCYGDGKTSERCYQLLKTIPLHSQILNKCNAY

SEQ ID NO: 12 - protein, 557 aa, S. cerevisiae
MKVDYEQLCKLYDDMCRTKNVQFSYGTAGFRTLAKNLDTVMFSTGILAVLRSLKLQGQYVGVMITASHNPYQDNGVKIVEPDGSMLLATWEPYAMQLANAASFATNFEEFRVELAKLIEHEKIDLNTTVVPHIVVGRDSRESSPYLLRCLTSSMASVFHAQVLDLGCVTTPQLHYITDLSNRRKLEGDTAPVATERDYYSFFIGAFNELFATYQLEKRLSVPKLFIDTANGIGGPQLKKLLASEDWDVPAEQVEVINDRSDVPELLNFECGADYVKTNQRLPKGLSPSSFDSLYCSFDGDADRVVFYYVDSGSKFHLLDGDKISTLFAKFLSKQLELAHLEHSLKIGVVQTAYANGSSTAYIKNTLHCPVSCTKTGVKHLHHEAATQYDIGIYFEANGHGTIIFSGKFHRTIKSELSKSKLNGDTLALRTLKCFSELINQTVGDAISDMLAVLATLAILKMSPMDWDEEYTDLPNKLVKCIVPDRSIFQTTDQERKLLNPVGLQDKIDLVVAKYPMGRSFVRASGTEDAVRVYAECKDSSKLGQFCDEVVEHVKASA

SEQ ID NO: 13 - protein, 477 aa, S. cerevisiae
MTDTKQLFIEAGQSQLFHNWESLSRKDQEELLSNLEQISSKRSPAKLLEDCQNAIKFSLANSSKDTGVEISPLPPTSYESLIGNSKKENEYWRLGLEAIGKGEVAVILMAGGQGTRLGSSQPKGCYDIGLPSKKSLFQIQAEKLIRLQDMVKDKKVEIPWYIMTSGPTRAATEAYFQEHNYFGLNKEQITFFNQGTLPAFDLTGKHFLMKDPVNLSQSPDGNGGLYRAIKENKLNEDFDRRGIKHVYMYCVDNVLSKIADPVFIGFAIKHGFELATKAVRKRDAHESVGLIATKNEKPCVIEYSEISNELAEAKDKDGLLKLRAGNIVNHYYLVDLLKRDLDQWCENMPYHIAKKKIPAYDSVTGKYTKPTEPNGIKLEQFIFDVFDTVPLNKFGCLEVDRCKEFSPLKNGPGSKNDNPETSRLAYLKLGTSWLEDAGAIVKDGVLVEVSSKLSYAGENLSQFKGKVFDRSGIVLEK

SEQ ID NO: 14 - protein, 496 aa, E. Coli
MSTTTQNIPWYRHLNRAQWRAFSAAWLGYLLDGFDFVLIALVLTEVQGEFGLTTVQAASLISAAFISRWFGGLMLGAMGDRYGRRLAMVTSIVLFSAGTLACGFAPGYITMFIARLVIGMGMAGEYGSSATYVIESWPKHLRNKASGFLISGFSVGAVVAAQVYSLVVPVWGWRALFFIGILPIIFALWLRKNIPEAEDWKEKHAGKAPVRTMVDILYRGEHRIANIVMTLAAATALWFCFAGNLQNAAIVAVLGLLCAAIFISFMVQSAGKRWPTGVMLMVVVLFAFLYSWPIQALLPTYLKTDLAYNPHTVANVLFFSGFGAAVGCCVGGFLGDWLGTRKAYVCSLLASQLLIIPVFAIGGANVWVLGLLLFFQQMLGQGIAGILPKLIGGYFDTDQRAAGLGFTYNVGALGGALAPIIGALIAQRLDLGTALASLSFSLTFVVILLIGLDMPSRVQRWLRPEALRTHDAIDGKPFSGAVPFGSAKNDLVKTKS

SEQ ID NO: 15 - protein, 297 aa, E. Coli
MATNLRGVMAALLTPFDQQQALDKASLRRLVQFNIQQGIDGLYVGGSTGEAFVQSLSEREQVLEIVAEEAKGKIKLIAHVGCVSTAESQQLAASAKRYGFDAVSAVTPFYYPFSFEEHCDHYRAIIDSADGLPMVVYNIPALSGVKLTLDQINTLVTLPGVGALKQTSGDLYQMEQIRREHPDLVLYNGYDEIFASGLLAGADGGIGSTYNIMGWRYQGIVKALKEGDIQTAQKLQTECNKVIDLLIKTGVFRGLKTVLHYMDVVSVPLCRKPFGPVDEKYLPELKALAQQLMQERG

SEQ ID NO: 16 - protein, 382 aa, E. Coli
MYALTQGRIFTGHEFLDDHAVVIADGLIKSVCPVAELPPEIEQRSLNGAILSPGFIDVQLNGCGGVQFNDTAEAVSVETLEIMQKANEKSGCTNYLPTLITTSDELMKQGVRVMREYLAKHPNQALGLHLEGPWLNLVKKGTHNPNFVRKPDAALVDFLCENADVITKVTLAPEMVPAEVISKLANAGIVVSAGHSNATLKEAKAGFRAGITFATHLYNAMPYITGREPGLAGAILDEADIYCGIIADGLHVDYANIRNAKRLKGDKLCLVTDATAPAGANIEQFIFAGKTIYYRNGLCVDENGTLSGSSLTMIEGVRNLVEHCGIALDEVLRMATLYPARAIGVEKRLGTLAAGKVANLTAFTPDFKITKTIVNGNEVVTQ

SEQ ID NO: 17 - protein, 229 aa, E. Coli
MSLLAQLDQKIAANGGLIVSCQPVPDSPLDKPEIVAAMALAAEQAGAVAIRIEGVANLQATRAVVSVPIIGIVKRDLEDSPVRITAYIEDVDALAQAGADIIAIDGTDRPRPVPVETLLARIHHHGLLAMTDCSTPEDGLACQKLGAEIIGTTLSGYTTPETPEEPDLALVKTLSDAGCRVIAEGRYNTPAQAADAMRHGAWAVTVGSAITRLEHICQWYNTAMKKAVL

SEQ ID NO: 18 - protein, 367 aa, E. Coli
MNLLTVSTDLISIFLFTTLFLFFARKVAKKVGLVDKPNFRKRHQGLIPLVGGISVYAGICFTFGIVDYYIPHASLYLACAGVLVFIGALDDRFDISVKIRATIQAAVGIVMMVFGKLYLSSLGYIFGSWEMVLGPFGYFLTLFAVWAAINAFNMVDGIDGLLGGLSCVSFAAIGMILWFDGQTSLAIWCFAMIAAILPYIMLNLGILGRRYKVFMGDAGSTLIGFTVIWILLETTQGKTHPISPVTALWIIAIPLMDMVAIMYRRLRKGMSPFSPDRQHIHHLIMRAGFTSRQAFVLITLAAALLASIGVLAEYSHFVPEWVMLVLFLLAFFLYGYCIKRAWKVARFIKRVKRRLRRNRGGSPNLTK

SEQ ID NO: 19 - DNA, 32 bp, pseB primer
gcagcatatgccaaatcatcaaaacatgctag

SEQ ID NO: 20 - DNA, 40 bp, pseB primer
gcaggaattctcataataatttcaacaaatcatcaggctc

SEQ ID NO: 21 - DNA, 43 bp, pseB primer
ccatttagccctagagttcgaagactttttcatcattcagccc

SEQ ID NO: 22 - DNA, 43 bp, pseB primer
gggctgaatgatgaaaaagtcttcgaactctagggctaaatgg

SEQ ID NO: 23 - DNA, 31 bp, pseC primer
gcagcatatgaaagagtttgcttatagcgag

SEQ ID NO: 24 - DNA, 36 bp, pseC primer
gcaggaattctcattctattttaaaactctcaaaag

SEQ ID NO: 25 - DNA, 47 bp, pseH primer
gcagcatatgaaaaaaaattattcttataaaaatatccaagcgattg

SEQ ID NO: 26 - DNA, 42 bp, pseH primer
gcaggaattcctaaagttttagaagagattgatcattatatc

SEQ ID NO: 27 - DNA, 34 bp, pseG primer
ggaccatatgaaagtgctttttagaagcgatagc

SEQ ID NO: 28 - DNA, 37 bp, pseG primer
ggacgaattctcaatacttatactccacttcataccc

SEQ ID NO: 29 - DNA, 31 bp, pseI primer
gcagcatatgttacaaccccctaaaattgtc

SEQ ID NO: 30 - DNA, 34 bp, pseI primer
gcaggaattcctacaatgagcgttctatatcatc

SEQ ID NO: 31 - DNA, 37 bp, pglF primer
gcagcatatgattttttataaaagcaaaagattagca

SEQ ID NO: 32 - DNA, 40 bp, pglF primer
gcaggaattcttatacaccttctttattgtgtttaaattc

SEQ ID NO: 33 - DNA, 47 bp, pglE primer
gcagcatatgagattttttctttctcctccgcacatgggtggtaatg

SEQ ID NO: 34 - DNA, 43 bp, pglE primer
gcaggaattcttaagcctttatgctctttaagatcagttttga

SEQ ID NO: 35 - DNA, 39 bp, pglD primer
gcagcatatggcaagaactgaaaaaatttatatttatgg

SEQ ID NO: 36 - DNA, 34 bp, pglD primer
gcaggaattcttacatcctttttgcaggtactcc

SEQ ID NO: 37 - DNA, 22 bp, colanic acid primer
gttatcgatgatcaggttgcgc

SEQ ID NO: 38 - DNA, 45 bp, colanic acid primer
gaagcagctccagcctacaccgccagcttgctgcaggctttatag

SEQ ID NO: 39 - DNA, 39 bp, colanic acid primer
ctaaggaggatattcattgtttatttatcactttggcag

SEQ ID NO: 40 - DNA, 23 bp, colanic acid primer
gtaataacctcacattatccctg

SEQ ID NO: 41 - DNA, 20 bp, colanic acid primer
gtgtaggctggagctgcttc

SEQ ID NO: 42 - DNA, 20 bp, colanic acid primer
gtgtaggctggagctgcttc

SEQ ID NO: 43 - DNA, 26 bp, pgaDABC primer
atgtattcaagtagcagaaaaaggtg

SEQ ID NO: 44 - DNA, 48 bp, pgaDABC primer
gaagcagctccagcctacacggttattgctgagtgctgattttagtgc

SEQ ID NO: 45 - DNA, 43 bp, pgaDABC primer
ctaaggaggatattcatgtctgggcgctgtacaataagctgcg

SEQ ID NO: 46 - DNA, 30 bp, pgaDABC primer
ttatgcccggactagcgctttttctgaaac

SEQ ID NO: 47 - DNA, 20 bp, pgaDABC primer
gtgtaggctggagctgcttc

SEQ ID NO: 48 - DNA, 20 bp, pgaDABC primer
atgggaattagccatggtcc